European Patent Application EP 4 803 638 A1, published September 9, 2026. Title: Methods for diagnosis and treating liver cancer. Applicant: ASOCIACIÓN CENTRO DE INVESTIGACIÓN COOPERATIVA EN BIOCIENCIAS-CIC bioGUNE. Application EP. The sequence listing filed with the application follows.

SEQUENCE LISTING (3 sequences)

SEQ ID NO: 1 - RNA, 19 nt, synthetic construct
  source 1..19: mol_type = other RNA; note = target region
tggccaagagcgataatgg

SEQ ID NO: 2 - DNA, 21 bp, synthetic construct
  misc_feature 1..19: note = RNA
  source 1..21: mol_type = other DNA; note = siRNA sense strand
  misc_feature 20..21: note = DNA
tggccaagagcgataatggtt

SEQ ID NO: 3 - DNA, 21 bp, synthetic construct
  misc_feature 1..19: note = RNA
  source 1..21: mol_type = other DNA; note = siRNA antisense strand
  misc_feature 20..21: note = DNA
ccattatcgctcttggccatt